European Patent Application EP 4 393 502 A2, published July 3, 2024. Title: ACETYLCHOLINE RECEPTOR INHIBITORY PEPTIDES AND USES THEREOF. Applicant: SKINMED CO., LTD. The sequence listing filed with the application follows.

SEQUENCE LISTING (606 sequences)

SEQ ID NO: 1 - protein, 8 aa, synthetic construct
  REGION 1..8: note = AchR binding peptide
KAKKIRQR

SEQ ID NO: 2 - protein, 8 aa, synthetic construct
  REGION 1..8: note = AchR binding peptide
KKRKGSAK

SEQ ID NO: 3 - protein, 8 aa, synthetic construct
  REGION 1..8: note = AchR binding peptide
RGKRQLGR

SEQ ID NO: 4 - protein, 8 aa, synthetic construct
  REGION 1..8: note = AchR binding peptide
KLKKFPVR

SEQ ID NO: 5 - protein, 8 aa, synthetic construct
  REGION 1..8: note = AchR binding peptide
RHKKSPWK

SEQ ID NO: 6 - protein, 8 aa, synthetic construct
  REGION 1..8: note = AchR binding peptide
RPRRTHIK

SEQ ID NO: 7 - protein, 8 aa, synthetic construct
  REGION 1..8: note = AchR binding peptide
KHKKLNQR

SEQ ID NO: 8 - protein, 8 aa, synthetic construct
  REGION 1..8: note = AchR binding peptide
RAKRMCCK

SEQ ID NO: 9 - protein, 8 aa, synthetic construct
  REGION 1..8: note = AchR binding peptide
RQRRNDMK

SEQ ID NO: 10 - protein, 8 aa, synthetic construct
  REGION 1..8: note = AchR binding peptide
KRKKDWWR

SEQ ID NO: 11 - protein, 8 aa, synthetic construct
  REGION 1..8: note = AchR binding peptide
RARKDAFK

SEQ ID NO: 12 - protein, 8 aa, synthetic construct
  REGION 1..8: note = AchR binding peptide
KWRREGFK

SEQ ID NO: 13 - protein, 8 aa, synthetic construct
  REGION 1..8: note = AchR binding peptide
RFRRGVRR

SEQ ID NO: 14 - protein, 8 aa, synthetic construct
  REGION 1..8: note = AchR binding peptide
KARRQEDK

SEQ ID NO: 15 - protein, 8 aa, synthetic construct
  REGION 1..8: note = AchR binding peptide
RFKRLCMK

SEQ ID NO: 16 - protein, 8 aa, synthetic construct
  REGION 1..8: note = AchR binding peptide
KLKRRSRR

SEQ ID NO: 17 - protein, 8 aa, synthetic construct
  REGION 1..8: note = AchR binding peptide
RPRRSLDR

SEQ ID NO: 18 - protein, 8 aa, synthetic construct
  REGION 1..8: note = AchR binding peptide
KHKKQNVR

SEQ ID NO: 19 - protein, 8 aa, synthetic construct
  REGION 1..8: note = AchR binding peptide
KFKRTEGR

SEQ ID NO: 20 - protein, 8 aa, synthetic construct
  REGION 1..8: note = AchR binding peptide
RGKKAVRK

SEQ ID NO: 21 - protein, 8 aa, synthetic construct
  REGION 1..8: note = AchR binding peptide
KFKKHGVK

SEQ ID NO: 22 - protein, 8 aa, synthetic construct
  REGION 1..8: note = AchR binding peptide
KTKKIHSK

SEQ ID NO: 23 - protein, 8 aa, synthetic construct
  REGION 1..8: note = AchR binding peptide
RDRKIHDK

SEQ ID NO: 24 - protein, 8 aa, synthetic construct
  REGION 1..8: note = AchR binding peptide
RPRRGHQK

SEQ ID NO: 25 - protein, 8 aa, synthetic construct
  REGION 1..8: note = AchR binding peptide
KTKKLYEK

SEQ ID NO: 26 - protein, 8 aa, synthetic construct
  REGION 1..8: note = AchR binding peptide
RQKKDNQK

SEQ ID NO: 27 - protein, 8 aa, synthetic construct
  REGION 1..8: note = AchR binding peptide
RQRKSMQR

SEQ ID NO: 28 - protein, 8 aa, synthetic construct
  REGION 1..8: note = AchR binding peptide
RGRRWFVK

SEQ ID NO: 29 - protein, 8 aa, synthetic construct
  REGION 1..8: note = AchR binding peptide
RNKRDENK

SEQ ID NO: 30 - protein, 8 aa, synthetic construct
  REGION 1..8: note = AchR binding peptide
RLRRWCVK

SEQ ID NO: 31 - protein, 8 aa, synthetic construct
  REGION 1..8: note = AchR binding peptide
RQKKPWVK

SEQ ID NO: 32 - protein, 8 aa, synthetic construct
  REGION 1..8: note = AchR binding peptide
RWKRSEQR

SEQ ID NO: 33 - protein, 8 aa, synthetic construct
  REGION 1..8: note = AchR binding peptide
RLKRAPGR

SEQ ID NO: 34 - protein, 8 aa, synthetic construct
  REGION 1..8: note = AchR binding peptide
KMRRAQGR

SEQ ID NO: 35 - protein, 8 aa, synthetic construct
  REGION 1..8: note = AchR binding peptide
KIKKAARR

SEQ ID NO: 36 - protein, 8 aa, synthetic construct
  REGION 1..8: note = AchR binding peptide
KNRKNLYR

SEQ ID NO: 37 - protein, 8 aa, synthetic construct
  REGION 1..8: note = AchR binding peptide
KCKKMTER

SEQ ID NO: 38 - protein, 8 aa, synthetic construct
  REGION 1..8: note = AchR binding peptide
KTRRVDLR

SEQ ID NO: 39 - protein, 8 aa, synthetic construct
  REGION 1..8: note = AchR binding peptide
KSRKWGWR

SEQ ID NO: 40 - protein, 8 aa, synthetic construct
  REGION 1..8: note = AchR binding peptide
KRRRFRWK

SEQ ID NO: 41 - protein, 8 aa, synthetic construct
  REGION 1..8: note = AchR binding peptide
KYKKQHTK

SEQ ID NO: 42 - protein, 8 aa, synthetic construct
  REGION 1..8: note = AchR binding peptide
RGRKKCGK

SEQ ID NO: 43 - protein, 8 aa, synthetic construct
  REGION 1..8: note = AchR binding peptide
KLRKQKLR

SEQ ID NO: 44 - protein, 8 aa, synthetic construct
  REGION 1..8: note = AchR binding peptide
RNRKIPLK

SEQ ID NO: 45 - protein, 8 aa, synthetic construct
  REGION 1..8: note = AchR binding peptide
RLRRRYRR

SEQ ID NO: 46 - protein, 8 aa, synthetic construct
  REGION 1..8: note = AchR binding peptide
KWRKRRIK

SEQ ID NO: 47 - protein, 8 aa, synthetic construct
  REGION 1..8: note = AchR binding peptide
KTKRMLAK

SEQ ID NO: 48 - protein, 8 aa, synthetic construct
  REGION 1..8: note = AchR binding peptide
KEKRAVHK

SEQ ID NO: 49 - protein, 8 aa, synthetic construct
  REGION 1..8: note = AchR binding peptide
RVRRDGHR

SEQ ID NO: 50 - protein, 8 aa, synthetic construct
  REGION 1..8: note = AchR binding peptide
RAKKCYHK

SEQ ID NO: 51 - protein, 8 aa, synthetic construct
  REGION 1..8: note = AchR binding peptide
KGKRDSNK

SEQ ID NO: 52 - protein, 8 aa, synthetic construct
  REGION 1..8: note = AchR binding peptide
KVRKSLWK

SEQ ID NO: 53 - protein, 8 aa, synthetic construct
  REGION 1..8: note = AchR binding peptide
RSKKSLYR

SEQ ID NO: 54 - protein, 8 aa, synthetic construct
  REGION 1..8: note = AchR binding peptide
RGKRGCER

SEQ ID NO: 55 - protein, 8 aa, synthetic construct
  REGION 1..8: note = AchR binding peptide
KQKKTGFR

SEQ ID NO: 56 - protein, 8 aa, synthetic construct
  REGION 1..8: note = AchR binding peptide
KYRRNLVR

SEQ ID NO: 57 - protein, 8 aa, synthetic construct
  REGION 1..8: note = AchR binding peptide
RIRRGSVR

SEQ ID NO: 58 - protein, 8 aa, synthetic construct
  REGION 1..8: note = AchR binding peptide
RSKRMNGK

SEQ ID NO: 59 - protein, 8 aa, synthetic construct
  REGION 1..8: note = AchR binding peptide
RHKKFIEK

SEQ ID NO: 60 - protein, 8 aa, synthetic construct
  REGION 1..8: note = AchR binding peptide
RIRRVSQR

SEQ ID NO: 61 - protein, 8 aa, synthetic construct
  REGION 1..8: note = AchR binding peptide
RPKKWMQK

SEQ ID NO: 62 - protein, 8 aa, synthetic construct
  REGION 1..8: note = AchR binding peptide
KERKHEAK

SEQ ID NO: 63 - protein, 8 aa, synthetic construct
  REGION 1..8: note = AchR binding peptide
KERKASAK

SEQ ID NO: 64 - protein, 8 aa, synthetic construct
  REGION 1..8: note = AchR binding peptide
KMRRIMYK

SEQ ID NO: 65 - protein, 8 aa, synthetic construct
  REGION 1..8: note = AchR binding peptide
KWKRNCTK

SEQ ID NO: 66 - protein, 8 aa, synthetic construct
  REGION 1..8: note = AchR binding peptide
RCKKNPEK

SEQ ID NO: 67 - protein, 8 aa, synthetic construct
  REGION 1..8: note = AchR binding peptide
KQRKPHGR

SEQ ID NO: 68 - protein, 8 aa, synthetic construct
  REGION 1..8: note = AchR binding peptide
KAKRGHFK

SEQ ID NO: 69 - protein, 8 aa, synthetic construct
  REGION 1..8: note = AchR binding peptide
KSKRHHEK

SEQ ID NO: 70 - protein, 8 aa, synthetic construct
  REGION 1..8: note = AchR binding peptide
KSRKHCNR

SEQ ID NO: 71 - protein, 8 aa, synthetic construct
  REGION 1..8: note = AchR binding peptide
RSKKINNK

SEQ ID NO: 72 - protein, 8 aa, synthetic construct
  REGION 1..8: note = AchR binding peptide
RVRRSWIR

SEQ ID NO: 73 - protein, 8 aa, synthetic construct
  REGION 1..8: note = AchR binding peptide
KSRRSAGK

SEQ ID NO: 74 - protein, 8 aa, synthetic construct
  REGION 1..8: note = AchR binding peptide
KMRKHDVR

SEQ ID NO: 75 - protein, 8 aa, synthetic construct
  REGION 1..8: note = AchR binding peptide
KGKKLSQR

SEQ ID NO: 76 - protein, 8 aa, synthetic construct
  REGION 1..8: note = AchR binding peptide
KWRREQFR

SEQ ID NO: 77 - protein, 8 aa, synthetic construct
  REGION 1..8: note = AchR binding peptide
KDKRWANR

SEQ ID NO: 78 - protein, 8 aa, synthetic construct
  REGION 1..8: note = AchR binding peptide
KHKRTAQR

SEQ ID NO: 79 - protein, 8 aa, synthetic construct
  REGION 1..8: note = AchR binding peptide
KPKREMHK

SEQ ID NO: 80 - protein, 8 aa, synthetic construct
  REGION 1..8: note = AchR binding peptide
RWKKNINK

SEQ ID NO: 81 - protein, 8 aa, synthetic construct
  REGION 1..8: note = AchR binding peptide
KWKKMMER

SEQ ID NO: 82 - protein, 8 aa, synthetic construct
  REGION 1..8: note = AchR binding peptide
RIRRWWVR

SEQ ID NO: 83 - protein, 8 aa, synthetic construct
  REGION 1..8: note = AchR binding peptide
RIRRHMYR

SEQ ID NO: 84 - protein, 8 aa, synthetic construct
  REGION 1..8: note = AchR binding peptide
KPKKPPAR

SEQ ID NO: 85 - protein, 8 aa, synthetic construct
  REGION 1..8: note = AchR binding peptide
RLKRGQFK

SEQ ID NO: 86 - protein, 8 aa, synthetic construct
  REGION 1..8: note = AchR binding peptide
KNKRTPVK

SEQ ID NO: 87 - protein, 8 aa, synthetic construct
  REGION 1..8: note = AchR binding peptide
KWRRAFGR

SEQ ID NO: 88 - protein, 8 aa, synthetic construct
  REGION 1..8: note = AchR binding peptide
KNKKCVGR

SEQ ID NO: 89 - protein, 8 aa, synthetic construct
  REGION 1..8: note = AchR binding peptide
RTRKCVLK

SEQ ID NO: 90 - protein, 8 aa, synthetic construct
  REGION 1..8: note = AchR binding peptide
KIKRDLYK

SEQ ID NO: 91 - protein, 8 aa, synthetic construct
  REGION 1..8: note = AchR binding peptide
REKRYMAR

SEQ ID NO: 92 - protein, 8 aa, synthetic construct
  REGION 1..8: note = AchR binding peptide
RVKKAETR

SEQ ID NO: 93 - protein, 8 aa, synthetic construct
  REGION 1..8: note = AchR binding peptide
RGRRGTMR

SEQ ID NO: 94 - protein, 8 aa, synthetic construct
  REGION 1..8: note = AchR binding peptide
RTKRWQLK

SEQ ID NO: 95 - protein, 8 aa, synthetic construct
  REGION 1..8: note = AchR binding peptide
RLRKSLGK

SEQ ID NO: 96 - protein, 8 aa, synthetic construct
  REGION 1..8: note = AchR binding peptide
RPKRNWAK

SEQ ID NO: 97 - protein, 8 aa, synthetic construct
  REGION 1..8: note = AchR binding peptide
KDRKVNSR

SEQ ID NO: 98 - protein, 8 aa, synthetic construct
  REGION 1..8: note = AchR binding peptide
KWRRNGQR

SEQ ID NO: 99 - protein, 8 aa, synthetic construct
  REGION 1..8: note = AchR binding peptide
RFKRMVWR

SEQ ID NO: 100 - protein, 8 aa, synthetic construct
  REGION 1..8: note = AchR binding peptide
KERKGAVR

SEQ ID NO: 101 - protein, 8 aa, synthetic construct
  REGION 1..8: note = AchR binding peptide
KTKRGSLK

SEQ ID NO: 102 - protein, 8 aa, synthetic construct
  REGION 1..8: note = AchR binding peptide
KTKRVDPK

SEQ ID NO: 103 - protein, 8 aa, synthetic construct
  REGION 1..8: note = AchR binding peptide
RARKLHNR

SEQ ID NO: 104 - protein, 8 aa, synthetic construct
  REGION 1..8: note = AchR binding peptide
RGKKPWWR

SEQ ID NO: 105 - protein, 8 aa, synthetic construct
  REGION 1..8: note = AchR binding peptide
KGKKYYQK

SEQ ID NO: 106 - protein, 8 aa, synthetic construct
  REGION 1..8: note = AchR binding peptide
RWRRSVIK

SEQ ID NO: 107 - protein, 8 aa, synthetic construct
  REGION 1..8: note = AchR binding peptide
RQKKDFLK

SEQ ID NO: 108 - protein, 8 aa, synthetic construct
  REGION 1..8: note = AchR binding peptide
RGRKPIWK

SEQ ID NO: 109 - protein, 8 aa, synthetic construct
  REGION 1..8: note = AchR binding peptide
KPRRPDTR

SEQ ID NO: 110 - protein, 8 aa, synthetic construct
  REGION 1..8: note = AchR binding peptide
KVKRLWNR

SEQ ID NO: 111 - protein, 8 aa, synthetic construct
  REGION 1..8: note = AchR binding peptide
KDRKGVYK

SEQ ID NO: 112 - protein, 8 aa, synthetic construct
  REGION 1..8: note = AchR binding peptide
RVKRFVPK

SEQ ID NO: 113 - protein, 8 aa, synthetic construct
  REGION 1..8: note = AchR binding peptide
KPKRDQSR

SEQ ID NO: 114 - protein, 8 aa, synthetic construct
  REGION 1..8: note = AchR binding peptide
KDKKQWGR

SEQ ID NO: 115 - protein, 8 aa, synthetic construct
  REGION 1..8: note = AchR binding peptide
RFRKMIPK

SEQ ID NO: 116 - protein, 8 aa, synthetic construct
  REGION 1..8: note = AchR binding peptide
KFRKHVCK

SEQ ID NO: 117 - protein, 8 aa, synthetic construct
  REGION 1..8: note = AchR binding peptide
RPKRSPSK

SEQ ID NO: 118 - protein, 8 aa, synthetic construct
  REGION 1..8: note = AchR binding peptide
RYKKVPAK

SEQ ID NO: 119 - protein, 8 aa, synthetic construct
  REGION 1..8: note = AchR binding peptide
RSRRCPVK

SEQ ID NO: 120 - protein, 8 aa, synthetic construct
  REGION 1..8: note = AchR binding peptide
RCKRCDNK

SEQ ID NO: 121 - protein, 8 aa, synthetic construct
  REGION 1..8: note = AchR binding peptide
RGKKQLSK

SEQ ID NO: 122 - protein, 8 aa, synthetic construct
  REGION 1..8: note = AchR binding peptide
KSKRPEGR

SEQ ID NO: 123 - protein, 8 aa, synthetic construct
  REGION 1..8: note = AchR binding peptide
KCRKTMGR

SEQ ID NO: 124 - protein, 8 aa, synthetic construct
  REGION 1..8: note = AchR binding peptide
RDRKNPVR

SEQ ID NO: 125 - protein, 8 aa, synthetic construct
  REGION 1..8: note = AchR binding peptide
KPKRSAPR

SEQ ID NO: 126 - protein, 8 aa, synthetic construct
  REGION 1..8: note = AchR binding peptide
KGKRTGCK

SEQ ID NO: 127 - protein, 8 aa, synthetic construct
  REGION 1..8: note = AchR binding peptide
RFRKPTDR

SEQ ID NO: 128 - protein, 8 aa, synthetic construct
  REGION 1..8: note = AchR binding peptide
RMKKFHTR

SEQ ID NO: 129 - protein, 8 aa, synthetic construct
  REGION 1..8: note = AchR binding peptide
KIKKYYWK

SEQ ID NO: 130 - protein, 8 aa, synthetic construct
  REGION 1..8: note = AchR binding peptide
RIKRNNCK

SEQ ID NO: 131 - protein, 8 aa, synthetic construct
  REGION 1..8: note = AchR binding peptide
RHKRMLWR

SEQ ID NO: 132 - protein, 8 aa, synthetic construct
  REGION 1..8: note = AchR binding peptide
KVRRVFLK

SEQ ID NO: 133 - protein, 8 aa, synthetic construct
  REGION 1..8: note = AchR binding peptide
KDKRPECK

SEQ ID NO: 134 - protein, 8 aa, synthetic construct
  REGION 1..8: note = AchR binding peptide
KTRRSACR

SEQ ID NO: 135 - protein, 8 aa, synthetic construct
  REGION 1..8: note = AchR binding peptide
KFRKGPYR

SEQ ID NO: 136 - protein, 8 aa, synthetic construct
  REGION 1..8: note = AchR binding peptide
KFKKSAPR

SEQ ID NO: 137 - protein, 8 aa, synthetic construct
  REGION 1..8: note = AchR binding peptide
KPRKIQGR

SEQ ID NO: 138 - protein, 8 aa, synthetic construct
  REGION 1..8: note = AchR binding peptide
KMRKGWDK

SEQ ID NO: 139 - protein, 8 aa, synthetic construct
  REGION 1..8: note = AchR binding peptide
KFRRQSTR

SEQ ID NO: 140 - protein, 8 aa, synthetic construct
  REGION 1..8: note = AchR binding peptide
KNRRADCR

SEQ ID NO: 141 - protein, 8 aa, synthetic construct
  REGION 1..8: note = AchR binding peptide
KNKRWVFK

SEQ ID NO: 142 - protein, 8 aa, synthetic construct
  REGION 1..8: note = AchR binding peptide
RCRKDTAR

SEQ ID NO: 143 - protein, 8 aa, synthetic construct
  REGION 1..8: note = AchR binding peptide
KARRVGTK

SEQ ID NO: 144 - protein, 8 aa, synthetic construct
  REGION 1..8: note = AchR binding peptide
KVKKIYYR

SEQ ID NO: 145 - protein, 8 aa, synthetic construct
  REGION 1..8: note = AchR binding peptide
KAKRDYLR

SEQ ID NO: 146 - protein, 8 aa, synthetic construct
  REGION 1..8: note = AchR binding peptide
KVKRLPYR

SEQ ID NO: 147 - protein, 8 aa, synthetic construct
  REGION 1..8: note = AchR binding peptide
RHRRANFR

SEQ ID NO: 148 - protein, 8 aa, synthetic construct
  REGION 1..8: note = AchR binding peptide
KPKKGGWK

SEQ ID NO: 149 - protein, 8 aa, synthetic construct
  REGION 1..8: note = AchR binding peptide
KEKRLYAR

SEQ ID NO: 150 - protein, 8 aa, synthetic construct
  REGION 1..8: note = AchR binding peptide
REKKQEVK

SEQ ID NO: 151 - protein, 8 aa, synthetic construct
  REGION 1..8: note = AchR binding peptide
KSRRAVFR

SEQ ID NO: 152 - protein, 8 aa, synthetic construct
  REGION 1..8: note = AchR binding peptide
RHRKYVDK

SEQ ID NO: 153 - protein, 8 aa, synthetic construct
  REGION 1..8: note = AchR binding peptide
RHKRWSGR

SEQ ID NO: 154 - protein, 8 aa, synthetic construct
  REGION 1..8: note = AchR binding peptide
RDRKFVQK

SEQ ID NO: 155 - protein, 8 aa, synthetic construct
  REGION 1..8: note = AchR binding peptide
RYRRWFYR

SEQ ID NO: 156 - protein, 8 aa, synthetic construct
  REGION 1..8: note = AchR binding peptide
RQRRMTPR

SEQ ID NO: 157 - protein, 8 aa, synthetic construct
  REGION 1..8: note = AchR binding peptide
RNKRMDGK

SEQ ID NO: 158 - protein, 8 aa, synthetic construct
  REGION 1..8: note = AchR binding peptide
RPKKHQER

SEQ ID NO: 159 - protein, 8 aa, synthetic construct
  REGION 1..8: note = AchR binding peptide
KKRKSLLR

SEQ ID NO: 160 - protein, 8 aa, synthetic construct
  REGION 1..8: note = AchR binding peptide
KIKRNVFK

SEQ ID NO: 161 - protein, 8 aa, synthetic construct
  REGION 1..8: note = AchR binding peptide
KYKREEYR

SEQ ID NO: 162 - protein, 8 aa, synthetic construct
  REGION 1..8: note = AchR binding peptide
KIRRVTNK

SEQ ID NO: 163 - protein, 8 aa, synthetic construct
  REGION 1..8: note = AchR binding peptide
KVKRVWGR

SEQ ID NO: 164 - protein, 8 aa, synthetic construct
  REGION 1..8: note = AchR binding peptide
RIKRDYCK

SEQ ID NO: 165 - protein, 8 aa, synthetic construct
  REGION 1..8: note = AchR binding peptide
RIRRAHDR

SEQ ID NO: 166 - protein, 8 aa, synthetic construct
  REGION 1..8: note = AchR binding peptide
RARKESHK

SEQ ID NO: 167 - protein, 8 aa, synthetic construct
  REGION 1..8: note = AchR binding peptide
RYKKQQYK

SEQ ID NO: 168 - protein, 8 aa, synthetic construct
  REGION 1..8: note = AchR binding peptide
KIKKLSQK

SEQ ID NO: 169 - protein, 8 aa, synthetic construct
  REGION 1..8: note = AchR binding peptide
KLKRAMLK

SEQ ID NO: 170 - protein, 8 aa, synthetic construct
  REGION 1..8: note = AchR binding peptide
KARKNSIR

SEQ ID NO: 171 - protein, 8 aa, synthetic construct
  REGION 1..8: note = AchR binding peptide
KERKLWWK

SEQ ID NO: 172 - protein, 8 aa, synthetic construct
  REGION 1..8: note = AchR binding peptide
KTRKQDHR

SEQ ID NO: 173 - protein, 8 aa, synthetic construct
  REGION 1..8: note = AchR binding peptide
RCKRFVGK

SEQ ID NO: 174 - protein, 8 aa, synthetic construct
  REGION 1..8: note = AchR binding peptide
KEKKLVWK

SEQ ID NO: 175 - protein, 8 aa, synthetic construct
  REGION 1..8: note = AchR binding peptide
KARRNSLK

SEQ ID NO: 176 - protein, 8 aa, synthetic construct
  REGION 1..8: note = AchR binding peptide
KMRRVAPR

SEQ ID NO: 177 - protein, 8 aa, synthetic construct
  REGION 1..8: note = AchR binding peptide
RAKKIMFR

SEQ ID NO: 178 - protein, 8 aa, synthetic construct
  REGION 1..8: note = AchR binding peptide
KTKKAAER

SEQ ID NO: 179 - protein, 8 aa, synthetic construct
  REGION 1..8: note = AchR binding peptide
RGKRHWHR

SEQ ID NO: 180 - protein, 8 aa, synthetic construct
  REGION 1..8: note = AchR binding peptide
RTKKENVK

SEQ ID NO: 181 - protein, 8 aa, synthetic construct
  REGION 1..8: note = AchR binding peptide
REKKYAYK

SEQ ID NO: 182 - protein, 8 aa, synthetic construct
  REGION 1..8: note = AchR binding peptide
KWRRELPR

SEQ ID NO: 183 - protein, 8 aa, synthetic construct
  REGION 1..8: note = AchR binding peptide
KSRRMWGR

SEQ ID NO: 184 - protein, 8 aa, synthetic construct
  REGION 1..8: note = AchR binding peptide
KCKKDNDK

SEQ ID NO: 185 - protein, 8 aa, synthetic construct
  REGION 1..8: note = AchR binding peptide
KDKKMPQR

SEQ ID NO: 186 - protein, 8 aa, synthetic construct
  REGION 1..8: note = AchR binding peptide
RHKRQQDK

SEQ ID NO: 187 - protein, 8 aa, synthetic construct
  REGION 1..8: note = AchR binding peptide
RLKKHCGK

SEQ ID NO: 188 - protein, 8 aa, synthetic construct
  REGION 1..8: note = AchR binding peptide
KARKQEVR

SEQ ID NO: 189 - protein, 8 aa, synthetic construct
  REGION 1..8: note = AchR binding peptide
KMRKFYSK

SEQ ID NO: 190 - protein, 8 aa, synthetic construct
  REGION 1..8: note = AchR binding peptide
KMRRWWLK

SEQ ID NO: 191 - protein, 8 aa, synthetic construct
  REGION 1..8: note = AchR binding peptide
KQKRQWAR

SEQ ID NO: 192 - protein, 8 aa, synthetic construct
  REGION 1..8: note = AchR binding peptide
RSRRGIGK

SEQ ID NO: 193 - protein, 8 aa, synthetic construct
  REGION 1..8: note = AchR binding peptide
KDKKTPCK

SEQ ID NO: 194 - protein, 8 aa, synthetic construct
  REGION 1..8: note = AchR binding peptide
RIRKITWR

SEQ ID NO: 195 - protein, 8 aa, synthetic construct
  REGION 1..8: note = AchR binding peptide
RHKRWEVR

SEQ ID NO: 196 - protein, 8 aa, synthetic construct
  REGION 1..8: note = AchR binding peptide
RFRRNFHK

SEQ ID NO: 197 - protein, 8 aa, synthetic construct
  REGION 1..8: note = AchR binding peptide
KWKRFSQR

SEQ ID NO: 198 - protein, 8 aa, synthetic construct
  REGION 1..8: note = AchR binding peptide
KYKKSFTK

SEQ ID NO: 199 - protein, 8 aa, synthetic construct
  REGION 1..8: note = AchR binding peptide
KTRKIVMK

SEQ ID NO: 200 - protein, 8 aa, synthetic construct
  REGION 1..8: note = AchR binding peptide
RTKKAYVK

SEQ ID NO: 201 - protein, 11 aa, synthetic construct
  REGION 1..11: note = AchR binding peptide
EDYKYRRQNYK

SEQ ID NO: 202 - protein, 11 aa, synthetic construct
  REGION 1..11: note = AchR binding peptide
GIWKFRRNQCK

SEQ ID NO: 203 - protein, 11 aa, synthetic construct
  REGION 1..11: note = AchR binding peptide
SPVRWKRLCLR

SEQ ID NO: 204 - protein, 11 aa, synthetic construct
  REGION 1..11: note = AchR binding peptide
ECYRNRKAYCR

SEQ ID NO: 205 - protein, 11 aa, synthetic construct
  REGION 1..11: note = AchR binding peptide
TQQRLKRVMEK

SEQ ID NO: 206 - protein, 11 aa, synthetic construct
  REGION 1..11: note = AchR binding peptide
PELKCKRMIGR

SEQ ID NO: 207 - protein, 11 aa, synthetic construct
  REGION 1..11: note = AchR binding peptide
WQMKTKKEIWK

SEQ ID NO: 208 - protein, 11 aa, synthetic construct
  REGION 1..11: note = AchR binding peptide
FGHRGKKEWAR

SEQ ID NO: 209 - protein, 11 aa, synthetic construct
  REGION 1..11: note = AchR binding peptide
ATCKPKRPWYK

SEQ ID NO: 210 - protein, 11 aa, synthetic construct
  REGION 1..11: note = AchR binding peptide
TSQKVRKMEAK

SEQ ID NO: 211 - protein, 11 aa, synthetic construct
  REGION 1..11: note = AchR binding peptide
GIPKYRRGCSR

SEQ ID NO: 212 - protein, 11 aa, synthetic construct
  REGION 1..11: note = AchR binding peptide
AYAKARRWGQK

SEQ ID NO: 213 - protein, 11 aa, synthetic construct
  REGION 1..11: note = AchR binding peptide
GGLKSKRLTTR

SEQ ID NO: 214 - protein, 11 aa, synthetic construct
  REGION 1..11: note = AchR binding peptide
GMWKVRKTVFR

SEQ ID NO: 215 - protein, 11 aa, synthetic construct
  REGION 1..11: note = AchR binding peptide
HTTRGKRCDPR

SEQ ID NO: 216 - protein, 11 aa, synthetic construct
  REGION 1..11: note = AchR binding peptide
VDVRNKKSNNR

SEQ ID NO: 217 - protein, 11 aa, synthetic construct
  REGION 1..11: note = AchR binding peptide
GLNRWRRCHHK

SEQ ID NO: 218 - protein, 11 aa, synthetic construct
  REGION 1..11: note = AchR binding peptide
LQSRSKKYSVK

SEQ ID NO: 219 - protein, 11 aa, synthetic construct
  REGION 1..11: note = AchR binding peptide
GWNRAKREESK

SEQ ID NO: 220 - protein, 11 aa, synthetic construct
  REGION 1..11: note = AchR binding peptide
SWQKCKKAEVR

SEQ ID NO: 221 - protein, 11 aa, synthetic construct
  REGION 1..11: note = AchR binding peptide
MVMKWKRWNQR

SEQ ID NO: 222 - protein, 11 aa, synthetic construct
  REGION 1..11: note = AchR binding peptide
MMMRHKRCQYR

SEQ ID NO: 223 - protein, 11 aa, synthetic construct
  REGION 1..11: note = AchR binding peptide
QTYRLKKPLQK

SEQ ID NO: 224 - protein, 11 aa, synthetic construct
  REGION 1..11: note = AchR binding peptide
SFWRERKNGFR

SEQ ID NO: 225 - protein, 11 aa, synthetic construct
  REGION 1..11: note = AchR binding peptide
RLERPRRELTK

SEQ ID NO: 226 - protein, 11 aa, synthetic construct
  REGION 1..11: note = AchR binding peptide
APWRLKRAPQR

SEQ ID NO: 227 - protein, 11 aa, synthetic construct
  REGION 1..11: note = AchR binding peptide
QGEKYRRTESK

SEQ ID NO: 228 - protein, 11 aa, synthetic construct
  REGION 1..11: note = AchR binding peptide
CIWKSKRSPAK

SEQ ID NO: 229 - protein, 11 aa, synthetic construct
  REGION 1..11: note = AchR binding peptide
AILKGKRIPNK

SEQ ID NO: 230 - protein, 11 aa, synthetic construct
  REGION 1..11: note = AchR binding peptide
PTLKWRKPVLR

SEQ ID NO: 231 - protein, 11 aa, synthetic construct
  REGION 1..11: note = AchR binding peptide
NNSRSKRFMNR

SEQ ID NO: 232 - protein, 11 aa, synthetic construct
  REGION 1..11: note = AchR binding peptide
LYMRCKKQAPR

SEQ ID NO: 233 - protein, 11 aa, synthetic construct
  REGION 1..11: note = AchR binding peptide
INYRCRKWVDK

SEQ ID NO: 234 - protein, 11 aa, synthetic construct
  REGION 1..11: note = AchR binding peptide
VMDRDRKWWWR

SEQ ID NO: 235 - protein, 11 aa, synthetic construct
  REGION 1..11: note = AchR binding peptide
NFTKLRKPGPR

SEQ ID NO: 236 - protein, 11 aa, synthetic construct
  REGION 1..11: note = AchR binding peptide
FIPKMRKCSPR

SEQ ID NO: 237 - protein, 11 aa, synthetic construct
  REGION 1..11: note = AchR binding peptide
TLWKVRKAYSR

SEQ ID NO: 238 - protein, 11 aa, synthetic construct
  REGION 1..11: note = AchR binding peptide
ESEKIKRLSTR

SEQ ID NO: 239 - protein, 11 aa, synthetic construct
  REGION 1..11: note = AchR binding peptide
LMTKNRRNSFR

SEQ ID NO: 240 - protein, 11 aa, synthetic construct
  REGION 1..11: note = AchR binding peptide
PEVKVRRHSMR

SEQ ID NO: 241 - protein, 11 aa, synthetic construct
  REGION 1..11: note = AchR binding peptide
AEVKDKKAYYK

SEQ ID NO: 242 - protein, 11 aa, synthetic construct
  REGION 1..11: note = AchR binding peptide
YYAKSKKYMVR

SEQ ID NO: 243 - protein, 11 aa, synthetic construct
  REGION 1..11: note = AchR binding peptide
LMDRTRRDMYK

SEQ ID NO: 244 - protein, 11 aa, synthetic construct
  REGION 1..11: note = AchR binding peptide
NMGRHKRPFLK

SEQ ID NO: 245 - protein, 11 aa, synthetic construct
  REGION 1..11: note = AchR binding peptide
WIYRGRKDVAK

SEQ ID NO: 246 - protein, 11 aa, synthetic construct
  REGION 1..11: note = AchR binding peptide
CYWKAKRYPMR

SEQ ID NO: 247 - protein, 11 aa, synthetic construct
  REGION 1..11: note = AchR binding peptide
IEDKGRRINPR

SEQ ID NO: 248 - protein, 11 aa, synthetic construct
  REGION 1..11: note = AchR binding peptide
VSTKIKKEPQR

SEQ ID NO: 249 - protein, 11 aa, synthetic construct
  REGION 1..11: note = AchR binding peptide
YPFKAKRPAEK

SEQ ID NO: 250 - protein, 11 aa, synthetic construct
  REGION 1..11: note = AchR binding peptide
SADRNKRHMTR

SEQ ID NO: 251 - protein, 11 aa, synthetic construct
  REGION 1..11: note = AchR binding peptide
SLYRQKRHDYK

SEQ ID NO: 252 - protein, 11 aa, synthetic construct
  REGION 1..11: note = AchR binding peptide
LPSRPKKPVPK

SEQ ID NO: 253 - protein, 11 aa, synthetic construct
  REGION 1..11: note = AchR binding peptide
PAWRCKRCQPK

SEQ ID NO: 254 - protein, 11 aa, synthetic construct
  REGION 1..11: note = AchR binding peptide
HHWRFKREMPR

SEQ ID NO: 255 - protein, 11 aa, synthetic construct
  REGION 1..11: note = AchR binding peptide
PACRSKRDWQK

SEQ ID NO: 256 - protein, 11 aa, synthetic construct
  REGION 1..11: note = AchR binding peptide
FICKSRKFYGK

SEQ ID NO: 257 - protein, 11 aa, synthetic construct
  REGION 1..11: note = AchR binding peptide
LEHKERKDDFR

SEQ ID NO: 258 - protein, 11 aa, synthetic construct
  REGION 1..11: note = AchR binding peptide
ANPKNRKDNLR

SEQ ID NO: 259 - protein, 11 aa, synthetic construct
  REGION 1..11: note = AchR binding peptide
FGVKYRRVICR

SEQ ID NO: 260 - protein, 11 aa, synthetic construct
  REGION 1..11: note = AchR binding peptide
HADKFRRFNMR

SEQ ID NO: 261 - protein, 11 aa, synthetic construct
  REGION 1..11: note = AchR binding peptide
PTIRVRKSDDR

SEQ ID NO: 262 - protein, 11 aa, synthetic construct
  REGION 1..11: note = AchR binding peptide
NLHKPKRDLPK

SEQ ID NO: 263 - protein, 11 aa, synthetic construct
  REGION 1..11: note = AchR binding peptide
IDGKWRKICTR

SEQ ID NO: 264 - protein, 11 aa, synthetic construct
  REGION 1..11: note = AchR binding peptide
SPFRAKRQDVR

SEQ ID NO: 265 - protein, 11 aa, synthetic construct
  REGION 1..11: note = AchR binding peptide
PLWKTRKIEPR

SEQ ID NO: 266 - protein, 11 aa, synthetic construct
  REGION 1..11: note = AchR binding peptide
PNYKWRKSRRR

SEQ ID NO: 267 - protein, 11 aa, synthetic construct
  REGION 1..11: note = AchR binding peptide
KTGRSKRHRWR

SEQ ID NO: 268 - protein, 11 aa, synthetic construct
  REGION 1..11: note = AchR binding peptide
GPDKSRRNLHR

SEQ ID NO: 269 - protein, 11 aa, synthetic construct
  REGION 1..11: note = AchR binding peptide
WCCKTKRAVMK

SEQ ID NO: 270 - protein, 11 aa, synthetic construct
  REGION 1..11: note = AchR binding peptide
QLLKMRKALSR

SEQ ID NO: 271 - protein, 11 aa, synthetic construct
  REGION 1..11: note = AchR binding peptide
PYLRSKRFPPR

SEQ ID NO: 272 - protein, 11 aa, synthetic construct
  REGION 1..11: note = AchR binding peptide
APHKWRKQEQR

SEQ ID NO: 273 - protein, 11 aa, synthetic construct
  REGION 1..11: note = AchR binding peptide
PPFKFRKPLGR

SEQ ID NO: 274 - protein, 11 aa, synthetic construct
  REGION 1..11: note = AchR binding peptide
CIMRVKRMWWK

SEQ ID NO: 275 - protein, 11 aa, synthetic construct
  REGION 1..11: note = AchR binding peptide
YILRDKKVPLK

SEQ ID NO: 276 - protein, 11 aa, synthetic construct
  REGION 1..11: note = AchR binding peptide
PWVRIRKMASR

SEQ ID NO: 277 - protein, 11 aa, synthetic construct
  REGION 1..11: note = AchR binding peptide
VADRQKKTAPK

SEQ ID NO: 278 - protein, 11 aa, synthetic construct
  REGION 1..11: note = AchR binding peptide
HHNRMKKQYHR

SEQ ID NO: 279 - protein, 11 aa, synthetic construct
  REGION 1..11: note = AchR binding peptide
EGAKYRRDGWR

SEQ ID NO: 280 - protein, 11 aa, synthetic construct
  REGION 1..11: note = AchR binding peptide
FWDRVKRNPSK

SEQ ID NO: 281 - protein, 11 aa, synthetic construct
  REGION 1..11: note = AchR binding peptide
TMWRQRKMSCK

SEQ ID NO: 282 - protein, 11 aa, synthetic construct
  REGION 1..11: note = AchR binding peptide
PDTRWKRVLFK

SEQ ID NO: 283 - protein, 11 aa, synthetic construct
  REGION 1..11: note = AchR binding peptide
HQQKCKKTTTK

SEQ ID NO: 284 - protein, 11 aa, synthetic construct
  REGION 1..11: note = AchR binding peptide
PWHKGKRDFDR

SEQ ID NO: 285 - protein, 11 aa, synthetic construct
  REGION 1..11: note = AchR binding peptide
VFVKWRRQMMR

SEQ ID NO: 286 - protein, 11 aa, synthetic construct
  REGION 1..11: note = AchR binding peptide
SQWKIRKRLIR

SEQ ID NO: 287 - protein, 11 aa, synthetic construct
  REGION 1..11: note = AchR binding peptide
EWHKVRRVYAK

SEQ ID NO: 288 - protein, 11 aa, synthetic construct
  REGION 1..11: note = AchR binding peptide
NAMRTKRMSFK

SEQ ID NO: 289 - protein, 11 aa, synthetic construct
  REGION 1..11: note = AchR binding peptide
PPFKFRKPLGR

SEQ ID NO: 290 - protein, 11 aa, synthetic construct
  REGION 1..11: note = AchR binding peptide
TSVKKRKQRLR

SEQ ID NO: 291 - protein, 11 aa, synthetic construct
  REGION 1..11: note = AchR binding peptide
PIDKFKRGMVR

SEQ ID NO: 292 - protein, 11 aa, synthetic construct
  REGION 1..11: note = AchR binding peptide
FVGRWKREYAK

SEQ ID NO: 293 - protein, 11 aa, synthetic construct
  REGION 1..11: note = AchR binding peptide
FNPKMRKVCLR

SEQ ID NO: 294 - protein, 11 aa, synthetic construct
  REGION 1..11: note = AchR binding peptide
NPGKTKRWLQR

SEQ ID NO: 295 - protein, 11 aa, synthetic construct
  REGION 1..11: note = AchR binding peptide
IMDKRRKPGCR

SEQ ID NO: 296 - protein, 11 aa, synthetic construct
  REGION 1..11: note = AchR binding peptide
ISDKAKRQHFK

SEQ ID NO: 297 - protein, 11 aa, synthetic construct
  REGION 1..11: note = AchR binding peptide
DVNKYRKHSHK

SEQ ID NO: 298 - protein, 11 aa, synthetic construct
  REGION 1..11: note = AchR binding peptide
LMLRGKRLTTK

SEQ ID NO: 299 - protein, 11 aa, synthetic construct
  REGION 1..11: note = AchR binding peptide
CSLRARKEEWR

SEQ ID NO: 300 - protein, 11 aa, synthetic construct
  REGION 1..11: note = AchR binding peptide
MNYRCKRVQER

SEQ ID NO: 301 - protein, 11 aa, synthetic construct
  REGION 1..11: note = AchR binding peptide
NGVRERKWQSK

SEQ ID NO: 302 - protein, 11 aa, synthetic construct
  REGION 1..11: note = AchR binding peptide
YTSRCKKQPRK

SEQ ID NO: 303 - protein, 11 aa, synthetic construct
  REGION 1..11: note = AchR binding peptide
QYNKGRKIHVR

SEQ ID NO: 304 - protein, 11 aa, synthetic construct
  REGION 1..11: note = AchR binding peptide
PEDRQRKTWFK

SEQ ID NO: 305 - protein, 11 aa, synthetic construct
  REGION 1..11: note = AchR binding peptide
IEMKPRKFGVK

SEQ ID NO: 306 - protein, 11 aa, synthetic construct
  REGION 1..11: note = AchR binding peptide
QRWKWRKSLAR

SEQ ID NO: 307 - protein, 11 aa, synthetic construct
  REGION 1..11: note = AchR binding peptide
VKHKERKCQRR

SEQ ID NO: 308 - protein, 11 aa, synthetic construct
  REGION 1..11: note = AchR binding peptide
QQDRPKRDIPK

SEQ ID NO: 309 - protein, 11 aa, synthetic construct
  REGION 1..11: note = AchR binding peptide
YPTKGKRCMIR

SEQ ID NO: 310 - protein, 11 aa, synthetic construct
  REGION 1..11: note = AchR binding peptide
RYAKHRKRQTR

SEQ ID NO: 311 - protein, 11 aa, synthetic construct
  REGION 1..11: note = AchR binding peptide
GYFRPRKETCK

SEQ ID NO: 312 - protein, 11 aa, synthetic construct
  REGION 1..11: note = AchR binding peptide
CFFKMRRCNTK

SEQ ID NO: 313 - protein, 11 aa, synthetic construct
  REGION 1..11: note = AchR binding peptide
QNDKDRKLSHR

SEQ ID NO: 314 - protein, 11 aa, synthetic construct
  REGION 1..11: note = AchR binding peptide
QVTKSKRVAFK

SEQ ID NO: 315 - protein, 11 aa, synthetic construct
  REGION 1..11: note = AchR binding peptide
VRAKHRKSSLR

SEQ ID NO: 316 - protein, 11 aa, synthetic construct
  REGION 1..11: note = AchR binding peptide
SHSRQRKTPLR

SEQ ID NO: 317 - protein, 11 aa, synthetic construct
  REGION 1..11: note = AchR binding peptide
DNGKIRRCLGK

SEQ ID NO: 318 - protein, 11 aa, synthetic construct
  REGION 1..11: note = AchR binding peptide
FLRRLKKVHWK

SEQ ID NO: 319 - protein, 11 aa, synthetic construct
  REGION 1..11: note = AchR binding peptide
FCRRSKKIGRR

SEQ ID NO: 320 - protein, 11 aa, synthetic construct
  REGION 1..11: note = AchR binding peptide
PAARTKRMYGR

SEQ ID NO: 321 - protein, 11 aa, synthetic construct
  REGION 1..11: note = AchR binding peptide
HETKPKKDGLR

SEQ ID NO: 322 - protein, 11 aa, synthetic construct
  REGION 1..11: note = AchR binding peptide
MGDRPRKWDSR

SEQ ID NO: 323 - protein, 11 aa, synthetic construct
  REGION 1..11: note = AchR binding peptide
HDTKCKKMYAK

SEQ ID NO: 324 - protein, 11 aa, synthetic construct
  REGION 1..11: note = AchR binding peptide
NVVRGRRLECR

SEQ ID NO: 325 - protein, 11 aa, synthetic construct
  REGION 1..11: note = AchR binding peptide
PADKGRREVMK

SEQ ID NO: 326 - protein, 11 aa, synthetic construct
  REGION 1..11: note = AchR binding peptide
AMMKYKKEFPK

SEQ ID NO: 327 - protein, 11 aa, synthetic construct
  REGION 1..11: note = AchR binding peptide
YIIRWKRQMTR

SEQ ID NO: 328 - protein, 11 aa, synthetic construct
  REGION 1..11: note = AchR binding peptide
SPWRIRRQNIR

SEQ ID NO: 329 - protein, 11 aa, synthetic construct
  REGION 1..11: note = AchR binding peptide
TCIKYRRAHTK

SEQ ID NO: 330 - protein, 11 aa, synthetic construct
  REGION 1..11: note = AchR binding peptide
GYDRARKGTLR

SEQ ID NO: 331 - protein, 11 aa, synthetic construct
  REGION 1..11: note = AchR binding peptide
MTLKHRRVYIK

SEQ ID NO: 332 - protein, 11 aa, synthetic construct
  REGION 1..11: note = AchR binding peptide
LFTRIKRLVCK

SEQ ID NO: 333 - protein, 11 aa, synthetic construct
  REGION 1..11: note = AchR binding peptide
DFSRDRRCLSK

SEQ ID NO: 334 - protein, 11 aa, synthetic construct
  REGION 1..11: note = AchR binding peptide
VWNKVKRWLER

SEQ ID NO: 335 - protein, 11 aa, synthetic construct
  REGION 1..11: note = AchR binding peptide
FPGKNRKYCSR

SEQ ID NO: 336 - protein, 11 aa, synthetic construct
  REGION 1..11: note = AchR binding peptide
YTSKNKRGCPR

SEQ ID NO: 337 - protein, 11 aa, synthetic construct
  REGION 1..11: note = AchR binding peptide
CACKQRRATSR

SEQ ID NO: 338 - protein, 11 aa, synthetic construct
  REGION 1..11: note = AchR binding peptide
IMERQRKSQHR

SEQ ID NO: 339 - protein, 11 aa, synthetic construct
  REGION 1..11: note = AchR binding peptide
SVLRCRKCSMK

SEQ ID NO: 340 - protein, 11 aa, synthetic construct
  REGION 1..11: note = AchR binding peptide
YPQKLRRTALK

SEQ ID NO: 341 - protein, 11 aa, synthetic construct
  REGION 1..11: note = AchR binding peptide
SSHKGKRAQSK

SEQ ID NO: 342 - protein, 11 aa, synthetic construct
  REGION 1..11: note = AchR binding peptide
DNPRFRKTILK

SEQ ID NO: 343 - protein, 11 aa, synthetic construct
  REGION 1..11: note = AchR binding peptide
AIIKFRKVQWK

SEQ ID NO: 344 - protein, 11 aa, synthetic construct
  REGION 1..11: note = AchR binding peptide
PYTRCRKEICK

SEQ ID NO: 345 - protein, 11 aa, synthetic construct
  REGION 1..11: note = AchR binding peptide
MNEKPKKNDQK

SEQ ID NO: 346 - protein, 11 aa, synthetic construct
  REGION 1..11: note = AchR binding peptide
LIGKFKKPFYR

SEQ ID NO: 347 - protein, 11 aa, synthetic construct
  REGION 1..11: note = AchR binding peptide
TWCKHKKLDMK

SEQ ID NO: 348 - protein, 11 aa, synthetic construct
  REGION 1..11: note = AchR binding peptide
DSNKVRKCSSK

SEQ ID NO: 349 - protein, 11 aa, synthetic construct
  REGION 1..11: note = AchR binding peptide
LPMKQRKCEFR

SEQ ID NO: 350 - protein, 11 aa, synthetic construct
  REGION 1..11: note = AchR binding peptide
EDVRVKRQTCR

SEQ ID NO: 351 - protein, 11 aa, synthetic construct
  REGION 1..11: note = AchR binding peptide
TQCKDRRVSDR

SEQ ID NO: 352 - protein, 11 aa, synthetic construct
  REGION 1..11: note = AchR binding peptide
IALKPKRVWLK

SEQ ID NO: 353 - protein, 11 aa, synthetic construct
  REGION 1..11: note = AchR binding peptide
GHQRGKREGSR

SEQ ID NO: 354 - protein, 11 aa, synthetic construct
  REGION 1..11: note = AchR binding peptide
NPFKYKKICPK

SEQ ID NO: 355 - protein, 11 aa, synthetic construct
  REGION 1..11: note = AchR binding peptide
NEARIKKCDVK

SEQ ID NO: 356 - protein, 11 aa, synthetic construct
  REGION 1..11: note = AchR binding peptide
YGLRMRKWYMK

SEQ ID NO: 357 - protein, 11 aa, synthetic construct
  REGION 1..11: note = AchR binding peptide
NFYKCRKLQCK

SEQ ID NO: 358 - protein, 11 aa, synthetic construct
  REGION 1..11: note = AchR binding peptide
MMTKYKKTCCK

SEQ ID NO: 359 - protein, 11 aa, synthetic construct
  REGION 1..11: note = AchR binding peptide
CNQKTKKIAEK

SEQ ID NO: 360 - protein, 11 aa, synthetic construct
  REGION 1..11: note = AchR binding peptide
ADIRMKKWYPK

SEQ ID NO: 361 - protein, 11 aa, synthetic construct
  REGION 1..11: note = AchR binding peptide
AWFRVKRSNCR

SEQ ID NO: 362 - protein, 11 aa, synthetic construct
  REGION 1..11: note = AchR binding peptide
NCDRTRKHWAR

SEQ ID NO: 363 - protein, 11 aa, synthetic construct
  REGION 1..11: note = AchR binding peptide
PHARTRKNITK

SEQ ID NO: 364 - protein, 11 aa, synthetic construct
  REGION 1..11: note = AchR binding peptide
VPTKMKKYETK

SEQ ID NO: 365 - protein, 11 aa, synthetic construct
  REGION 1..11: note = AchR binding peptide
AYPKFRKTFNR

SEQ ID NO: 366 - protein, 11 aa, synthetic construct
  REGION 1..11: note = AchR binding peptide
QQLRLRKLCGK

SEQ ID NO: 367 - protein, 11 aa, synthetic construct
  REGION 1..11: note = AchR binding peptide
MFMRNKKLAWR

SEQ ID NO: 368 - protein, 11 aa, synthetic construct
  REGION 1..11: note = AchR binding peptide
GGAKNKKVVSR

SEQ ID NO: 369 - protein, 11 aa, synthetic construct
  REGION 1..11: note = AchR binding peptide
HDPRHKKTPTK

SEQ ID NO: 370 - protein, 11 aa, synthetic construct
  REGION 1..11: note = AchR binding peptide
QVHRNKRYTDR

SEQ ID NO: 371 - protein, 11 aa, synthetic construct
  REGION 1..11: note = AchR binding peptide
YGTRPKKYVSK

SEQ ID NO: 372 - protein, 11 aa, synthetic construct
  REGION 1..11: note = AchR binding peptide
CTWRGRRPHDK

SEQ ID NO: 373 - protein, 11 aa, synthetic construct
  REGION 1..11: note = AchR binding peptide
SWAKARKLVHR

SEQ ID NO: 374 - protein, 11 aa, synthetic construct
  REGION 1..11: note = AchR binding peptide
PLFKSRRAYVR

SEQ ID NO: 375 - protein, 11 aa, synthetic construct
  REGION 1..11: note = AchR binding peptide
CVMRCRRSEDK

SEQ ID NO: 376 - protein, 11 aa, synthetic construct
  REGION 1..11: note = AchR binding peptide
WWHKHRRAQSK

SEQ ID NO: 377 - protein, 11 aa, synthetic construct
  REGION 1..11: note = AchR binding peptide
LNSKPRRVEFK

SEQ ID NO: 378 - protein, 11 aa, synthetic construct
  REGION 1..11: note = AchR binding peptide
VPYRHRRMQFK

SEQ ID NO: 379 - protein, 11 aa, synthetic construct
  REGION 1..11: note = AchR binding peptide
GIAKSKRNAGR

SEQ ID NO: 380 - protein, 11 aa, synthetic construct
  REGION 1..11: note = AchR binding peptide
DPEKWRKFYDR

SEQ ID NO: 381 - protein, 11 aa, synthetic construct
  REGION 1..11: note = AchR binding peptide
PGARCRKQDVK

SEQ ID NO: 382 - protein, 11 aa, synthetic construct
  REGION 1..11: note = AchR binding peptide
HEQRPKKGQQK

SEQ ID NO: 383 - protein, 11 aa, synthetic construct
  REGION 1..11: note = AchR binding peptide
TCDRARKESFR

SEQ ID NO: 384 - protein, 11 aa, synthetic construct
  REGION 1..11: note = AchR binding peptide
MHQRERRNFVK

SEQ ID NO: 385 - protein, 11 aa, synthetic construct
  REGION 1..11: note = AchR binding peptide
FITRFRKMGEK

SEQ ID NO: 386 - protein, 11 aa, synthetic construct
  REGION 1..11: note = AchR binding peptide
PNWKVRRFGDK

SEQ ID NO: 387 - protein, 11 aa, synthetic construct
  REGION 1..11: note = AchR binding peptide
TAAKWKKIIMK

SEQ ID NO: 388 - protein, 11 aa, synthetic construct
  REGION 1..11: note = AchR binding peptide
CLWRLRKDNGR

SEQ ID NO: 389 - protein, 11 aa, synthetic construct
  REGION 1..11: note = AchR binding peptide
AHIKSRKVWSR

SEQ ID NO: 390 - protein, 11 aa, synthetic construct
  REGION 1..11: note = AchR binding peptide
NLVKSKKVEEK

SEQ ID NO: 391 - protein, 11 aa, synthetic construct
  REGION 1..11: note = AchR binding peptide
PDSRLKKHEAK

SEQ ID NO: 392 - protein, 11 aa, synthetic construct
  REGION 1..11: note = AchR binding peptide
EHVKLKRLDFR

SEQ ID NO: 393 - protein, 11 aa, synthetic construct
  REGION 1..11: note = AchR binding peptide
PALRMRRWCQK

SEQ ID NO: 394 - protein, 11 aa, synthetic construct
  REGION 1..11: note = AchR binding peptide
HLEKHRRCEFK

SEQ ID NO: 395 - protein, 11 aa, synthetic construct
  REGION 1..11: note = AchR binding peptide
CQAKTRKAEDR

SEQ ID NO: 396 - protein, 11 aa, synthetic construct
  REGION 1..11: note = AchR binding peptide
QNMRMKRFIQR

SEQ ID NO: 397 - protein, 11 aa, synthetic construct
  REGION 1..11: note = AchR binding peptide
CPYRIRRGPGK

SEQ ID NO: 398 - protein, 11 aa, synthetic construct
  REGION 1..11: note = AchR binding peptide
DIYKGKRTLVK

SEQ ID NO: 399 - protein, 11 aa, synthetic construct
  REGION 1..11: note = AchR binding peptide
EICKNRKPANR

SEQ ID NO: 400 - protein, 11 aa, synthetic construct
  REGION 1..11: note = AchR binding peptide
QGMKLKRIWSK

SEQ ID NO: 401 - protein, 14 aa, synthetic construct
  REGION 1..14: note = AchR binding peptide
ALGRTKRLHMRVHV

SEQ ID NO: 402 - protein, 14 aa, synthetic construct
  REGION 1..14: note = AchR binding peptide
SFYKERKCQFRSGL

SEQ ID NO: 403 - protein, 14 aa, synthetic construct
  REGION 1..14: note = AchR binding peptide
SGVRYRKWWIRSVV

SEQ ID NO: 404 - protein, 14 aa, synthetic construct
  REGION 1..14: note = AchR binding peptide
MPQKLKKLDIRNHN

SEQ ID NO: 405 - protein, 14 aa, synthetic construct
  REGION 1..14: note = AchR binding peptide
NEDRGKRPHIRVLG

SEQ ID NO: 406 - protein, 14 aa, synthetic construct
  REGION 1..14: note = AchR binding peptide
EFVKLRKARLRGPQ

SEQ ID NO: 407 - protein, 14 aa, synthetic construct
  REGION 1..14: note = AchR binding peptide
EGDKFRRHDIKYNF

SEQ ID NO: 408 - protein, 14 aa, synthetic construct
  REGION 1..14: note = AchR binding peptide
PICRWKRAPFKWYF

SEQ ID NO: 409 - protein, 14 aa, synthetic construct
  REGION 1..14: note = AchR binding peptide
NCNRFRRTIVRHCH

SEQ ID NO: 410 - protein, 14 aa, synthetic construct
  REGION 1..14: note = AchR binding peptide
AHGKDRRYVEKLEV

SEQ ID NO: 411 - protein, 14 aa, synthetic construct
  REGION 1..14: note = AchR binding peptide
FMQKCKKWWDRAVF

SEQ ID NO: 412 - protein, 14 aa, synthetic construct
  REGION 1..14: note = AchR binding peptide
DPPKKRKSLLRRVS

SEQ ID NO: 413 - protein, 14 aa, synthetic construct
  REGION 1..14: note = AchR binding peptide
YCTRIRREGMKGSE

SEQ ID NO: 414 - protein, 14 aa, synthetic construct
  REGION 1..14: note = AchR binding peptide
FPGKSKKQWHRLWP

SEQ ID NO: 415 - protein, 14 aa, synthetic construct
  REGION 1..14: note = AchR binding peptide
YEPRFKRPYGKWCH

SEQ ID NO: 416 - protein, 14 aa, synthetic construct
  REGION 1..14: note = AchR binding peptide
DYLRSRKMEERFQE

SEQ ID NO: 417 - protein, 14 aa, synthetic construct
  REGION 1..14: note = AchR binding peptide
VGPKFRKNHRRQNR

SEQ ID NO: 418 - protein, 14 aa, synthetic construct
  REGION 1..14: note = AchR binding peptide
EYQKCKKPSFRLTM

SEQ ID NO: 419 - protein, 14 aa, synthetic construct
  REGION 1..14: note = AchR binding peptide
YMKKKRKSLLRTSL

SEQ ID NO: 420 - protein, 14 aa, synthetic construct
  REGION 1..14: note = AchR binding peptide
CCFKLKKAYNKGPF

SEQ ID NO: 421 - protein, 14 aa, synthetic construct
  REGION 1..14: note = AchR binding peptide
NPMKLRKAETKHNV

SEQ ID NO: 422 - protein, 14 aa, synthetic construct
  REGION 1..14: note = AchR binding peptide
HSLKTRKSAFKSNT

SEQ ID NO: 423 - protein, 14 aa, synthetic construct
  REGION 1..14: note = AchR binding peptide
QYHKVRKLWFRVEP

SEQ ID NO: 424 - protein, 14 aa, synthetic construct
  REGION 1..14: note = AchR binding peptide
FVRKKRKSLLRDTR

SEQ ID NO: 425 - protein, 14 aa, synthetic construct
  REGION 1..14: note = AchR binding peptide
CFQRKRKSLLRVLR

SEQ ID NO: 426 - protein, 14 aa, synthetic construct
  REGION 1..14: note = AchR binding peptide
VPMKYRRCGNRQSN

SEQ ID NO: 427 - protein, 14 aa, synthetic construct
  REGION 1..14: note = AchR binding peptide
RARKKRKSLLRRQV

SEQ ID NO: 428 - protein, 14 aa, synthetic construct
  REGION 1..14: note = AchR binding peptide
PNGKVRKRIRRRYF

SEQ ID NO: 429 - protein, 14 aa, synthetic construct
  REGION 1..14: note = AchR binding peptide
CASKPRRTYLRAAN

SEQ ID NO: 430 - protein, 14 aa, synthetic construct
  REGION 1..14: note = AchR binding peptide
WAHKCKKPGQRIPP

SEQ ID NO: 431 - protein, 14 aa, synthetic construct
  REGION 1..14: note = AchR binding peptide
LSDKKRKSLLRYDY

SEQ ID NO: 432 - protein, 14 aa, synthetic construct
  REGION 1..14: note = AchR binding peptide
CATRGKKVFSKRTM

SEQ ID NO: 433 - protein, 14 aa, synthetic construct
  REGION 1..14: note = AchR binding peptide
LRQRSKRVLEKLRP

SEQ ID NO: 434 - protein, 14 aa, synthetic construct
  REGION 1..14: note = AchR binding peptide
LGWKKRKSLLRRHV

SEQ ID NO: 435 - protein, 14 aa, synthetic construct
  REGION 1..14: note = AchR binding peptide
LQCKYRRGSDKQPQ

SEQ ID NO: 436 - protein, 14 aa, synthetic construct
  REGION 1..14: note = AchR binding peptide
AFSRIKRGVLKLLS

SEQ ID NO: 437 - protein, 14 aa, synthetic construct
  REGION 1..14: note = AchR binding peptide
SNVKRKRGRCKPYR

SEQ ID NO: 438 - protein, 14 aa, synthetic construct
  REGION 1..14: note = AchR binding peptide
TVVKSRKCSVRYNW

SEQ ID NO: 439 - protein, 14 aa, synthetic construct
  REGION 1..14: note = AchR binding peptide
DDVKQRKKHPRVQT

SEQ ID NO: 440 - protein, 14 aa, synthetic construct
  REGION 1..14: note = AchR binding peptide
ASPKGRRPTFRPQH

SEQ ID NO: 441 - protein, 14 aa, synthetic construct
  REGION 1..14: note = AchR binding peptide
GWLKAKRFPSRPPT

SEQ ID NO: 442 - protein, 14 aa, synthetic construct
  REGION 1..14: note = AchR binding peptide
ETNRTRKQCYKTTF

SEQ ID NO: 443 - protein, 14 aa, synthetic construct
  REGION 1..14: note = AchR binding peptide
FTHKNRRDSLRVWM

SEQ ID NO: 444 - protein, 14 aa, synthetic construct
  REGION 1..14: note = AchR binding peptide
PPFRLRKPLWRPQR

SEQ ID NO: 445 - protein, 14 aa, synthetic construct
  REGION 1..14: note = AchR binding peptide
PGNRMKKYQNRVHG

SEQ ID NO: 446 - protein, 14 aa, synthetic construct
  REGION 1..14: note = AchR binding peptide
SAHKKRKQTLRCSE

SEQ ID NO: 447 - protein, 14 aa, synthetic construct
  REGION 1..14: note = AchR binding peptide
LYEKYKKHNNREDD

SEQ ID NO: 448 - protein, 14 aa, synthetic construct
  REGION 1..14: note = AchR binding peptide
PHCRQKKFWIRCGT

SEQ ID NO: 449 - protein, 14 aa, synthetic construct
  REGION 1..14: note = AchR binding peptide
VAFKTRRRVQRQSG

SEQ ID NO: 450 - protein, 14 aa, synthetic construct
  REGION 1..14: note = AchR binding peptide
VFDKFRKTENRGVI

SEQ ID NO: 451 - protein, 14 aa, synthetic construct
  REGION 1..14: note = AchR binding peptide
NHHKTKRCSVRFNI

SEQ ID NO: 452 - protein, 14 aa, synthetic construct
  REGION 1..14: note = AchR binding peptide
GTFKWRKSGARQYL

SEQ ID NO: 453 - protein, 14 aa, synthetic construct
  REGION 1..14: note = AchR binding peptide
HCLRTKKLINKICS

SEQ ID NO: 454 - protein, 14 aa, synthetic construct
  REGION 1..14: note = AchR binding peptide
FFLRCRRLLGKVQV

SEQ ID NO: 455 - protein, 14 aa, synthetic construct
  REGION 1..14: note = AchR binding peptide
HFPRARRFEHRCML

SEQ ID NO: 456 - protein, 14 aa, synthetic construct
  REGION 1..14: note = AchR binding peptide
QISKLKRPSYRGDD

SEQ ID NO: 457 - protein, 14 aa, synthetic construct
  REGION 1..14: note = AchR binding peptide
EEIKQKKLHLRVWF

SEQ ID NO: 458 - protein, 14 aa, synthetic construct
  REGION 1..14: note = AchR binding peptide
SLPKWRKGGDRVFT

SEQ ID NO: 459 - protein, 14 aa, synthetic construct
  REGION 1..14: note = AchR binding peptide
HVYKNRRVWGKGWP

SEQ ID NO: 460 - protein, 14 aa, synthetic construct
  REGION 1..14: note = AchR binding peptide
EDLRCKKLELRSVI

SEQ ID NO: 461 - protein, 14 aa, synthetic construct
  REGION 1..14: note = AchR binding peptide
THDKCKKHNDKQAH

SEQ ID NO: 462 - protein, 14 aa, synthetic construct
  REGION 1..14: note = AchR binding peptide
YPERPRKLQDKSYS

SEQ ID NO: 463 - protein, 14 aa, synthetic construct
  REGION 1..14: note = AchR binding peptide
CPWRNRKAMIKGII

SEQ ID NO: 464 - protein, 14 aa, synthetic construct
  REGION 1..14: note = AchR binding peptide
HEIKQKKYFHRGHD

SEQ ID NO: 465 - protein, 14 aa, synthetic construct
  REGION 1..14: note = AchR binding peptide
CLEKLRKAVHRQRR

SEQ ID NO: 466 - protein, 14 aa, synthetic construct
  REGION 1..14: note = AchR binding peptide
YISKSKKTAGRWFW

SEQ ID NO: 467 - protein, 14 aa, synthetic construct
  REGION 1..14: note = AchR binding peptide
VTWKFRKAEKRWGY

SEQ ID NO: 468 - protein, 14 aa, synthetic construct
  REGION 1..14: note = AchR binding peptide
YSSKSRKLSPRTPR

SEQ ID NO: 469 - protein, 14 aa, synthetic construct
  REGION 1..14: note = AchR binding peptide
CVNRVKKSDSKGTW

SEQ ID NO: 470 - protein, 14 aa, synthetic construct
  REGION 1..14: note = AchR binding peptide
DHERERRLWSRFPF

SEQ ID NO: 471 - protein, 14 aa, synthetic construct
  REGION 1..14: note = AchR binding peptide
PLIKVKRGVGKLWN

SEQ ID NO: 472 - protein, 14 aa, synthetic construct
  REGION 1..14: note = AchR binding peptide
TGCRCKRSMYKNLH

SEQ ID NO: 473 - protein, 14 aa, synthetic construct
  REGION 1..14: note = AchR binding peptide
WTCRMRKYQLRTSE

SEQ ID NO: 474 - protein, 14 aa, synthetic construct
  REGION 1..14: note = AchR binding peptide
IAIRPRKMTLKIHP

SEQ ID NO: 475 - protein, 14 aa, synthetic construct
  REGION 1..14: note = AchR binding peptide
QIPKQKKQEQRAIS

SEQ ID NO: 476 - protein, 14 aa, synthetic construct
  REGION 1..14: note = AchR binding peptide
QMGKFKKISLKNTF

SEQ ID NO: 477 - protein, 14 aa, synthetic construct
  REGION 1..14: note = AchR binding peptide
VLIKQRKWQDRSCS

SEQ ID NO: 478 - protein, 14 aa, synthetic construct
  REGION 1..14: note = AchR binding peptide
FITKSRRQQFRNQG

SEQ ID NO: 479 - protein, 14 aa, synthetic construct
  REGION 1..14: note = AchR binding peptide
QQFKYRRECVKYGS

SEQ ID NO: 480 - protein, 14 aa, synthetic construct
  REGION 1..14: note = AchR binding peptide
MEGREKKSYNKGEN

SEQ ID NO: 481 - protein, 14 aa, synthetic construct
  REGION 1..14: note = AchR binding peptide
PTWRHRRYCAKDIG

SEQ ID NO: 482 - protein, 14 aa, synthetic construct
  REGION 1..14: note = AchR binding peptide
HMCRSKRVAWKNLI

SEQ ID NO: 483 - protein, 14 aa, synthetic construct
  REGION 1..14: note = AchR binding peptide
SYLKCKRSDYKEVP

SEQ ID NO: 484 - protein, 14 aa, synthetic construct
  REGION 1..14: note = AchR binding peptide
HTFKLRKLCQKLFE

SEQ ID NO: 485 - protein, 14 aa, synthetic construct
  REGION 1..14: note = AchR binding peptide
QLVKLRKLARRVSY

SEQ ID NO: 486 - protein, 14 aa, synthetic construct
  REGION 1..14: note = AchR binding peptide
SEVRPKKDHSRLFI

SEQ ID NO: 487 - protein, 14 aa, synthetic construct
  REGION 1..14: note = AchR binding peptide
FLEKCRKFIIRVST

SEQ ID NO: 488 - protein, 14 aa, synthetic construct
  REGION 1..14: note = AchR binding peptide
PETRHRKMFIRDFW

SEQ ID NO: 489 - protein, 14 aa, synthetic construct
  REGION 1..14: note = AchR binding peptide
EWCKNKRWHSREYP

SEQ ID NO: 490 - protein, 14 aa, synthetic construct
  REGION 1..14: note = AchR binding peptide
LWNRYKKLLMRIFW

SEQ ID NO: 491 - protein, 14 aa, synthetic construct
  REGION 1..14: note = AchR binding peptide
CWCRQRKCFHKPWI

SEQ ID NO: 492 - protein, 14 aa, synthetic construct
  REGION 1..14: note = AchR binding peptide
NLERTKKHGLKGYM

SEQ ID NO: 493 - protein, 14 aa, synthetic construct
  REGION 1..14: note = AchR binding peptide
EGGRIKRPNYRGDG

SEQ ID NO: 494 - protein, 14 aa, synthetic construct
  REGION 1..14: note = AchR binding peptide
PVLKLRKGRVRAQP

SEQ ID NO: 495 - protein, 14 aa, synthetic construct
  REGION 1..14: note = AchR binding peptide
SISRLRKAHQKFIP

SEQ ID NO: 496 - protein, 14 aa, synthetic construct
  REGION 1..14: note = AchR binding peptide
EWHKHRREMVRWGP

SEQ ID NO: 497 - protein, 14 aa, synthetic construct
  REGION 1..14: note = AchR binding peptide
WSAKGRRMGCKSTM

SEQ ID NO: 498 - protein, 14 aa, synthetic construct
  REGION 1..14: note = AchR binding peptide
PNGKVRKRIRRRYF

SEQ ID NO: 499 - protein, 14 aa, synthetic construct
  REGION 1..14: note = AchR binding peptide
PCWKFRRAQMKWGI

SEQ ID NO: 500 - protein, 14 aa, synthetic construct
  REGION 1..14: note = AchR binding peptide
LEERPKKHCAKNHC

SEQ ID NO: 501 - protein, 14 aa, synthetic construct
  REGION 1..14: note = AchR binding peptide
QPWRQKKFWCRCWG

SEQ ID NO: 502 - protein, 14 aa, synthetic construct
  REGION 1..14: note = AchR binding peptide
IMVKIRRCPARPLC

SEQ ID NO: 503 - protein, 14 aa, synthetic construct
  REGION 1..14: note = AchR binding peptide
NDWKLRKDFWRNHF

SEQ ID NO: 504 - protein, 14 aa, synthetic construct
  REGION 1..14: note = AchR binding peptide
ASVRDRKMGYKSDG

SEQ ID NO: 505 - protein, 14 aa, synthetic construct
  REGION 1..14: note = AchR binding peptide
YYEKIRRGEIKIAE

SEQ ID NO: 506 - protein, 14 aa, synthetic construct
  REGION 1..14: note = AchR binding peptide
DLVRKRKTMLRQLV

SEQ ID NO: 507 - protein, 14 aa, synthetic construct
  REGION 1..14: note = AchR binding peptide
DLSKVRRGHGKNDI

SEQ ID NO: 508 - protein, 14 aa, synthetic construct
  REGION 1..14: note = AchR binding peptide
ESYRLRRGTDKEQW

SEQ ID NO: 509 - protein, 14 aa, synthetic construct
  REGION 1..14: note = AchR binding peptide
YITKFRKFLMKDQF

SEQ ID NO: 510 - protein, 14 aa, synthetic construct
  REGION 1..14: note = AchR binding peptide
AWAKYKKVQPKHHT

SEQ ID NO: 511 - protein, 14 aa, synthetic construct
  REGION 1..14: note = AchR binding peptide
TWLRGRRWPDKQPQ

SEQ ID NO: 512 - protein, 14 aa, synthetic construct
  REGION 1..14: note = AchR binding peptide
ALPRVRKDSHREEI

SEQ ID NO: 513 - protein, 14 aa, synthetic construct
  REGION 1..14: note = AchR binding peptide
CLFKYRKSCVRLCG

SEQ ID NO: 514 - protein, 14 aa, synthetic construct
  REGION 1..14: note = AchR binding peptide
LQNRMRKIYWKTFD

SEQ ID NO: 515 - protein, 14 aa, synthetic construct
  REGION 1..14: note = AchR binding peptide
NDPRLRKHNHRCCT

SEQ ID NO: 516 - protein, 14 aa, synthetic construct
  REGION 1..14: note = AchR binding peptide
YGSKQRRFEEKICG

SEQ ID NO: 517 - protein, 14 aa, synthetic construct
  REGION 1..14: note = AchR binding peptide
CGHKNKKWHNRMDP

SEQ ID NO: 518 - protein, 14 aa, synthetic construct
  REGION 1..14: note = AchR binding peptide
YGIRDRRPMTKHTQ

SEQ ID NO: 519 - protein, 14 aa, synthetic construct
  REGION 1..14: note = AchR binding peptide
TPLKSRKYWNKHAY

SEQ ID NO: 520 - protein, 14 aa, synthetic construct
  REGION 1..14: note = AchR binding peptide
FLYKAKKALMRDSL

SEQ ID NO: 521 - protein, 14 aa, synthetic construct
  REGION 1..14: note = AchR binding peptide
CDDKPKKTVVKLTW

SEQ ID NO: 522 - protein, 14 aa, synthetic construct
  REGION 1..14: note = AchR binding peptide
MHPRPRKMSHKMSC

SEQ ID NO: 523 - protein, 14 aa, synthetic construct
  REGION 1..14: note = AchR binding peptide
PGERLKKEDHRASG

SEQ ID NO: 524 - protein, 14 aa, synthetic construct
  REGION 1..14: note = AchR binding peptide
GAQRARKPVLRAVG

SEQ ID NO: 525 - protein, 14 aa, synthetic construct
  REGION 1..14: note = AchR binding peptide
MQEKCRRCVFKGNI

SEQ ID NO: 526 - protein, 14 aa, synthetic construct
  REGION 1..14: note = AchR binding peptide
YVDRWRRMQYKLSI

SEQ ID NO: 527 - protein, 14 aa, synthetic construct
  REGION 1..14: note = AchR binding peptide
WVDRSRKFEDRNCL

SEQ ID NO: 528 - protein, 14 aa, synthetic construct
  REGION 1..14: note = AchR binding peptide
IVNRAKRSQIRFDV

SEQ ID NO: 529 - protein, 14 aa, synthetic construct
  REGION 1..14: note = AchR binding peptide
IHPRYKRHQARSCC

SEQ ID NO: 530 - protein, 14 aa, synthetic construct
  REGION 1..14: note = AchR binding peptide
EHSKHRKDLFRMVG

SEQ ID NO: 531 - protein, 14 aa, synthetic construct
  REGION 1..14: note = AchR binding peptide
YTPKFRRIFWRIID

SEQ ID NO: 532 - protein, 14 aa, synthetic construct
  REGION 1..14: note = AchR binding peptide
TITRVKRASHKTPS

SEQ ID NO: 533 - protein, 14 aa, synthetic construct
  REGION 1..14: note = AchR binding peptide
VDSREKKWRQKCQC

SEQ ID NO: 534 - protein, 14 aa, synthetic construct
  REGION 1..14: note = AchR binding peptide
YWFRIKRAHAKGCP

SEQ ID NO: 535 - protein, 14 aa, synthetic construct
  REGION 1..14: note = AchR binding peptide
NDHRMRRSVDRGET

SEQ ID NO: 536 - protein, 14 aa, synthetic construct
  REGION 1..14: note = AchR binding peptide
PFDRARRDLHRIMM

SEQ ID NO: 537 - protein, 14 aa, synthetic construct
  REGION 1..14: note = AchR binding peptide
QVVRLRRGKNRGTV

SEQ ID NO: 538 - protein, 14 aa, synthetic construct
  REGION 1..14: note = AchR binding peptide
TNQRPRRETAKTIE

SEQ ID NO: 539 - protein, 14 aa, synthetic construct
  REGION 1..14: note = AchR binding peptide
FHHRHKRIATKHPA

SEQ ID NO: 540 - protein, 14 aa, synthetic construct
  REGION 1..14: note = AchR binding peptide
EHCKWKKMFDKEGE

SEQ ID NO: 541 - protein, 14 aa, synthetic construct
  REGION 1..14: note = AchR binding peptide
FFYRLRRCLTRWWV

SEQ ID NO: 542 - protein, 14 aa, synthetic construct
  REGION 1..14: note = AchR binding peptide
LQCKYRRGSDKTVV

SEQ ID NO: 543 - protein, 14 aa, synthetic construct
  REGION 1..14: note = AchR binding peptide
QTMKFKRCCNKEMV

SEQ ID NO: 544 - protein, 14 aa, synthetic construct
  REGION 1..14: note = AchR binding peptide
CSYKLRRCDMRLWG

SEQ ID NO: 545 - protein, 14 aa, synthetic construct
  REGION 1..14: note = AchR binding peptide
MHIKMKREQVKDEE

SEQ ID NO: 546 - protein, 14 aa, synthetic construct
  REGION 1..14: note = AchR binding peptide
AVWRNRKDNVKASE

SEQ ID NO: 547 - protein, 14 aa, synthetic construct
  REGION 1..14: note = AchR binding peptide
ADHRAKKTLSKFWT

SEQ ID NO: 548 - protein, 14 aa, synthetic construct
  REGION 1..14: note = AchR binding peptide
MMARCRRIMCRSFN

SEQ ID NO: 549 - protein, 14 aa, synthetic construct
  REGION 1..14: note = AchR binding peptide
PFGKFKRLENKDEC

SEQ ID NO: 550 - protein, 14 aa, synthetic construct
  REGION 1..14: note = AchR binding peptide
YLSRTKRWLARYVE

SEQ ID NO: 551 - protein, 14 aa, synthetic construct
  REGION 1..14: note = AchR binding peptide
HTLKPKRLYPRPSE

SEQ ID NO: 552 - protein, 14 aa, synthetic construct
  REGION 1..14: note = AchR binding peptide
VVIKCRKWTHKMDH

SEQ ID NO: 553 - protein, 14 aa, synthetic construct
  REGION 1..14: note = AchR binding peptide
FHTKLRKPIPKIDM

SEQ ID NO: 554 - protein, 14 aa, synthetic construct
  REGION 1..14: note = AchR binding peptide
ENIKSRKYFVKLTW

SEQ ID NO: 555 - protein, 14 aa, synthetic construct
  REGION 1..14: note = AchR binding peptide
AWTRFRRFQCKGMS

SEQ ID NO: 556 - protein, 14 aa, synthetic construct
  REGION 1..14: note = AchR binding peptide
IVPRDRKQALRWTN

SEQ ID NO: 557 - protein, 14 aa, synthetic construct
  REGION 1..14: note = AchR binding peptide
CMLRWKRWHMRFNP

SEQ ID NO: 558 - protein, 14 aa, synthetic construct
  REGION 1..14: note = AchR binding peptide
FDMRDRRPNARVMP

SEQ ID NO: 559 - protein, 14 aa, synthetic construct
  REGION 1..14: note = AchR binding peptide
QIAKLKRDQMKEAW

SEQ ID NO: 560 - protein, 14 aa, synthetic construct
  REGION 1..14: note = AchR binding peptide
LTSRCKKTFQKNSE

SEQ ID NO: 561 - protein, 14 aa, synthetic construct
  REGION 1..14: note = AchR binding peptide
MAAKWKKDGMKSHY

SEQ ID NO: 562 - protein, 14 aa, synthetic construct
  REGION 1..14: note = AchR binding peptide
ANWRTRRDLAKEHV

SEQ ID NO: 563 - protein, 14 aa, synthetic construct
  REGION 1..14: note = AchR binding peptide
PFTKMRKQFQRMSA

SEQ ID NO: 564 - protein, 14 aa, synthetic construct
  REGION 1..14: note = AchR binding peptide
QINRVKKSDAKFCT

SEQ ID NO: 565 - protein, 14 aa, synthetic construct
  REGION 1..14: note = AchR binding peptide
YLVKLRRFWAKIDM

SEQ ID NO: 566 - protein, 14 aa, synthetic construct
  REGION 1..14: note = AchR binding peptide
EYVKAKRTPWKYVV

SEQ ID NO: 567 - protein, 14 aa, synthetic construct
  REGION 1..14: note = AchR binding peptide
AMCREKRFPYRAIY

SEQ ID NO: 568 - protein, 14 aa, synthetic construct
  REGION 1..14: note = AchR binding peptide
MGLRARKYEDKTLH

SEQ ID NO: 569 - protein, 14 aa, synthetic construct
  REGION 1..14: note = AchR binding peptide
FHMKSKKDGDKFVM

SEQ ID NO: 570 - protein, 14 aa, synthetic construct
  REGION 1..14: note = AchR binding peptide
CIFKFKKNMFKGYS

SEQ ID NO: 571 - protein, 14 aa, synthetic construct
  REGION 1..14: note = AchR binding peptide
LDTKNRRGASKWDY

SEQ ID NO: 572 - protein, 14 aa, synthetic construct
  REGION 1..14: note = AchR binding peptide
VTGKGRRVTFRCMN

SEQ ID NO: 573 - protein, 14 aa, synthetic construct
  REGION 1..14: note = AchR binding peptide
QLGKQKREATREYV

SEQ ID NO: 574 - protein, 14 aa, synthetic construct
  REGION 1..14: note = AchR binding peptide
SSGKWKRPHAKYIV

SEQ ID NO: 575 - protein, 14 aa, synthetic construct
  REGION 1..14: note = AchR binding peptide
TCHKTKRSIMRATS

SEQ ID NO: 576 - protein, 14 aa, synthetic construct
  REGION 1..14: note = AchR binding peptide
MIGKCRKCGTKCYA

SEQ ID NO: 577 - protein, 14 aa, synthetic construct
  REGION 1..14: note = AchR binding peptide
FQPKSRRAETKHSY

SEQ ID NO: 578 - protein, 14 aa, synthetic construct
  REGION 1..14: note = AchR binding peptide
PDLKFRKHQDRTAI

SEQ ID NO: 579 - protein, 14 aa, synthetic construct
  REGION 1..14: note = AchR binding peptide
YNARVKREGIKNIT

SEQ ID NO: 580 - protein, 14 aa, synthetic construct
  REGION 1..14: note = AchR binding peptide
QGIRPRKHLQRMPN

SEQ ID NO: 581 - protein, 14 aa, synthetic construct
  REGION 1..14: note = AchR binding peptide
GPCRPRRHSIRLLW

SEQ ID NO: 582 - protein, 14 aa, synthetic construct
  REGION 1..14: note = AchR binding peptide
FYLRERRHQLKTEF

SEQ ID NO: 583 - protein, 14 aa, synthetic construct
  REGION 1..14: note = AchR binding peptide
NMARSRKNECKYIA

SEQ ID NO: 584 - protein, 14 aa, synthetic construct
  REGION 1..14: note = AchR binding peptide
DMDKVKKWVWRSFP

SEQ ID NO: 585 - protein, 14 aa, synthetic construct
  REGION 1..14: note = AchR binding peptide
VLPKERRWLTRFLI

SEQ ID NO: 586 - protein, 14 aa, synthetic construct
  REGION 1..14: note = AchR binding peptide
YEHRHKRFFHKDMP

SEQ ID NO: 587 - protein, 14 aa, synthetic construct
  REGION 1..14: note = AchR binding peptide
HGHKPRRWIYRMPM

SEQ ID NO: 588 - protein, 14 aa, synthetic construct
  REGION 1..14: note = AchR binding peptide
DGIRDKKCCWRDLI

SEQ ID NO: 589 - protein, 14 aa, synthetic construct
  REGION 1..14: note = AchR binding peptide
ELVKHRRLDFRDPM

SEQ ID NO: 590 - protein, 14 aa, synthetic construct
  REGION 1..14: note = AchR binding peptide
VHHKLRRVHLRLDV

SEQ ID NO: 591 - protein, 14 aa, synthetic construct
  REGION 1..14: note = AchR binding peptide
GINRGRKVSPKDEQ

SEQ ID NO: 592 - protein, 14 aa, synthetic construct
  REGION 1..14: note = AchR binding peptide
NGYRARKENLKFPE

SEQ ID NO: 593 - protein, 14 aa, synthetic construct
  REGION 1..14: note = AchR binding peptide
AAYRARKIVEKSGW

SEQ ID NO: 594 - protein, 14 aa, synthetic construct
  REGION 1..14: note = AchR binding peptide
WAPRDRRNMGRDPA

SEQ ID NO: 595 - protein, 14 aa, synthetic construct
  REGION 1..14: note = AchR binding peptide
IEDKSKRFNCKECG

SEQ ID NO: 596 - protein, 14 aa, synthetic construct
  REGION 1..14: note = AchR binding peptide
IEMRYRRDCSRFVN

SEQ ID NO: 597 - protein, 14 aa, synthetic construct
  REGION 1..14: note = AchR binding peptide
QQIKYKRPTYRMVC

SEQ ID NO: 598 - protein, 14 aa, synthetic construct
  REGION 1..14: note = AchR binding peptide
LPWRERRNGGRSSE

SEQ ID NO: 599 - protein, 14 aa, synthetic construct
  REGION 1..14: note = AchR binding peptide
PQTRYRKYFYRPQM

SEQ ID NO: 600 - protein, 14 aa, synthetic construct
  REGION 1..14: note = AchR binding peptide
HMCRWRRQINKGVS

SEQ ID NO: 601 - protein, 11 aa, synthetic construct
  REGION 1..11: note = AchR binding peptide
RRRRRRRRRRR

SEQ ID NO: 602 - protein, 11 aa, synthetic construct
  REGION 1..11: note = AchR binding peptide
GGGRKKRRQRR

SEQ ID NO: 603 - protein, 11 aa, synthetic construct
  REGION 1..11: note = AchR binding peptide
GGRKKRRQRRR

SEQ ID NO: 604 - protein, 14 aa, synthetic construct
  REGION 1..14: note = AchR binding peptide
GGGRKKRRQRRRGG

SEQ ID NO: 605 - protein, 14 aa, synthetic construct
  REGION 1..14: note = AchR binding peptide
GGRKKRRQRRRGGG

SEQ ID NO: 606 - protein, 11 aa, synthetic construct
  REGION 1..11: note = AchR binding peptide
GGGRRRRRRRR